European Patent Specification EP 3 332 801 B1, published September 13, 2023. Title: DNA VACCINES AND METHODS FOR THE PREVENTION OF TRANSPLANTATION REJECTION. Applicant: Loma Linda University. The sequence listing filed with the application follows.

SEQUENCE LISTING (3 sequences)

SEQ ID NO: 1 - DNA, 1638 bp, Homo sapiens
atgtacaggatgcaactcctgtcttgcattgcactaagtcttgcacttgtcacaaacagtgcacctacttacgcgtttctccatgcaacagacctgctgccggcgtgtgatggagaaaggcccactttggcgtttctgcaagatgttatgaacattttacttcagtatgtggtgaaaagtttcgatagatcaaccaaagtgattgatttccattatcctaatgagcttctccaagaatataattgggaattggcagaccaaccacaaaatttggaggaaattttgatgcattgccaaacaactctaaaatatgcaattaaaacagggcatcctagatacttcaatcaactttctactggtttggatatggttggattagcagcagactggctgacatcaacagcaaatactaacatgttcacctatgaaattgctccagtatttgtgcttttggaatatgtcacactaaagaaaatgagagaaatcattggctggccagggggctctggcgatgggatattttctcccggtggcgccatatctaacatgtatgccatgatgatcgcacgctttaagatgttcccagaagtcaaggagaaaggaatggctgctcttcccaggctcattgccttcacgtctgaacatagtcatttttctctcaagaagggagctgcagccttagggattggaagagacagcgtgattctgattaaatgtgatgagagagggaaaatgattccatctgatcttgaaagaaggattcttgaagccaaacagaaagggtttgttcctttcctcgtgagtgccacagctggaaccaccgtgtacggagcatttgaccccctcttagctgtcgctgacatttgcaaaaagtataagatctggatgcatgtggatgcagcttggggtgggggattactgatgtcccgaaaacacaagtggaaactgagtggcgtggagagggccaactctgtgacgtggaatccacacaagatgatgggagtccctttgcagtggtctgctctcctggttagagaagagggattgatgcagaattgcaaccaaatgcatgcctcctacctctttcagcaagataaacattatgacctgtcctatgacactggagacaaggccttacagtgcggacgccacgttgatgtttttaaactatggctgatgtggagggcaaaggggactaccgggtttgaagcgcatgttgataaatgtttggagttggcagagtatttatacaacatcataaaaaaccgagaaggatatgagatggtgtttgatgggaagcctgaggacacaaatgtctgcttctggtacattcctccaagcttgcgtactctggaagacaatgaagagagaatgagtcgcctctcgaaggtggctccagtgattaaagccagaatgatggagtatggaaccacaatggtcagctaccaacccttgggagacaaggtcaatttcttccgcatggtcatctcaaacccagcggcaactcaccaagacattgacttcctgattgaagaaatagaacgccttggacaagatttataataaccttgctcaccaagctgttccacttctctaggtagcgacctcgagcggccgctcgagggggggcccggtacc

SEQ ID NO: 2 - DNA, 579 bp, Homo sapiens
atggacgggtccggggagcagcccagaggcggggggcccaccagctctgagcagatcatgaagacaggggcccttttgcttcagggtttcatccaggatcgagcagggcgaatggggggggaggcacccgagctggccctggacccggtgcctcaggatgcgtccaccaagaagctgagcgagtgtctcaagcgcatcggggacgaactggacagtaacatggagctgcagaggatgattgccgccgtggacacagactccccccgagaggtctttttccgagtggcagctgacatgttttctgacggcaacttcaactggggccgggttgtcgcccttttctactttgccagcaaactggtgctcaaggccctgtgcaccaaggtgccggaactgatcagaaccatcatgggctggacattggacttcctccgggagcggctgttgggctggatccaagaccagggtggttgggacggcctcctctcctactttgggacgcccacgtggcagaccgtgaccatctttgtggcgggagtgctcaccgcctcgctcaccatctggaagaagatgggctga

SEQ ID NO: 3 - DNA, 619 bp, Encephalomyocarditis virus
tctagataatacgactcactatagggcgaattccccctctccctcccccccccctaacgttactggccgaagccgcttggaataaggccggtgtgcgtttgtctatatgttattttccaccatattgccgtcttttggcaatgtgagggcccggaaacctggccctgtcttcttgacgagcattcctaggggtctttcccctctcgccaaaggaatgcaaggtctgttgaatgtcgtgaaggaagcagttcctctggaagcttcttgaagacaaacaacgtctgtagcgaccctttgcaggcagcggaaccccccacctggcgacaggtgcctctgcggccaaaagccaggtgtataagatacacctgcaaaggcggcacaaccccagtgccacgttgtgagttggaatagttgtggaaagagtcaaatggctctcctcaagcgtattcaacaaggggctgaaggatgcccagaaggtaccccattgtatgggatctgatctggggcctcggtgcacatgctttacatgtgtttagtcgaggttaaaaaacgtctaggccccccaaccacggggacgtggttttcctttgaaaaacacgattattatattgcctctaga